European Patent Specification EP 3 884 026 B1, published June 26, 2024. Title: Detergent Composition. Applicant: Unilever. The sequence listing filed with the application follows.

SEQUENCE LISTING (1 sequence)

SEQ ID NO: 1 - protein, 309 aa, Vulcanisaeta moutnovskia
MPLDPAVGRVLEELNKVMPQMTKIPLSEFRKMFRAFFASQSRRSIYKVYDITIPGTEAKIPVRIYVPREGTDLGILVYFHGGGFVLGDVETYDPLCRELAVACDCVVVSVDYRLAPEHKFPAAVIDSFDSTKWVLEHAREINGDPEKVAVGGDSAGGNLAAVVAIMARDQGLKPSLKYQVLINPFVGVDPASYTIREYSTGLFLEREAMAFFNKAYLRSPADAFDPRFSPILIDNLSNLPPALIITSEYDPLRDSAETYAAKLAESGVPTIVVRFNGVTHGFYGFPIPHAKAAVGLIGTTLRQAFYGKY